European Patent Application EP 4 310 179 A1, published January 24, 2024. Title: A MICROORGANISM OF CORYNEBACTERIUM GENUS HAVING ENHANCED L-ARGININE OR L-CITRULLINE PRODUCTIVITY AND A METHOD FOR PRODUCING L-ARGININE OR L-CITRULLINE USING THE SAME. Applicant: DAESANG CORPORATION. Application EP. The sequence listing filed with the application follows.

SEQUENCE LISTING (12 sequences)

SEQ ID NO: 1 - DNA, 1176 bp, Corynebacterium sp.
  source 1..1176: mol_type = genomic DNA
atgagcacgctggaaacttggccacaggtcattattaatacgtacggcaccccaccagttgagctggtgtccggcaagggcgcaaccgtcactgatgaccagggcaatgtctacatcgacttgctcgcgggcatcgcagtcaacgcgttgggccacgcccacccggcgatcatcgaggcggtcaccaaccagatcggccaacttggtcacgtctcaaacttgttcgcatccaggcccgtcgtcgaggtcgccgaggagctcatcaagcgtttttcgcttgacgacgccaccctcgccgcgcaaacccgggttttcttctgcaactcgggcgccgaagcaaacgaggctgctttcaagattgcacgcttgactggtcgttcccggattctggctgcagttcatggtttccacggccgcaccatgggttccctcgcgctgactggccagccagacaagcgtgaagcgttcctgccaatgccaagcggtgtggagttctacccttacggcgacaccgattacttgcgcaaaatggtagaaaccaacccaacggatgtggctgctatcttcctcgagccaatccagggtgaaacgggcgttgttccagcacctgaaggattcctcaaggcagtgcgcgagctgtgcgatgagtacggcatcttgatgatcaccgatgaagtccagactggcgttggccgtaccggcgatttctttgcacatcagcacgatggcgttgttcccgatgtggtgaccatggccaagggacttggcggcggtcttcccatcggtgcttgtttggccactggccgtgcagctgaattgatgaccccaggcaagcacggcaccactttcggtggcaacccagttgcttgtgcagctgccaaggcagtgctgtctgttgtcgatgacgctttctgcgcagaagttgcccgcaagggcgagctgttcaaggaacttcttgccaaggttgacggcgttgtagacgtccgtggcaggggcttgatgttgggcgtggtgctggagcgcgacgtcgcaaagcaagctgttcttgatggttttaagcacggcgttattttgaatgcaccggcggacaacattatccgtttgaccccgccgctggtgatcaccgacgaagaaatcgcagacgcagtcaaggctattgccgagacaatcgcataa

SEQ ID NO: 2 - protein, 391 aa, Corynebacterium sp.
MSTLETWPQVIINTYGTPPVELVSGKGATVTDDQGNVYIDLLAGIAVNALGHAHPAIIEAVTNQIGQLGHVSNLFASRPVVEVAEELIKRFSLDDATLAAQTRVFFCNSGAEANEAAFKIARLTGRSRILAAVHGFHGRTMGSLALTGQPDKREAFLPMPSGVEFYPYGDTDYLRKMVETNPTDVAAIFLEPIQGETGVVPAPEGFLKAVRELCDEYGILMITDEVQTGVGRTGDFFAHQHDGVVPDVVTMAKGLGGGLPIGACLATGRAAELMTPGKHGTTFGGNPVACAAAKAVLSVVDDAFCAEVARKGELFKELLAKVDGVVDVRGRGLMLGVVLERDVAKQAVLDGFKHGVILNAPADNIIRLTPPLVITDEEIADAVKAIAETIA

SEQ ID NO: 3 - DNA, 1176 bp, synthetic construct
  source 1..1176: mol_type = other DNA
atgagcacgctggaaacttggccacaggtcattattaatacgtacggcaccccaccagttgagctggtgtccggcaagggcgcaaccgtcactgatgaccagggcaatgtctacatcgacttgctcgcgggcatcgcagtcaacgcgttgggccacgcccacccggcgatcatcgaggcggtcaccaaccagatcggccaacttggtcacgtctcaaacttgttcgcatccaggcccgtcgtcgaggtcgccgaggagctcatcaagcgtttttcgcttgacgacgccaccctcgccgcgcaaacccgggttttcttctgcaactcgggcgccgaagcaaacgaggctgctttcaagattgcacgcttgactggtcgttcccggattctgactgcagttcatggtttccacggccgcaccatgggttccctcgcgctgactggccagccagacaagcgtgaagcgttcctgccaatgccaagcggtgtggagttctacccttacggcgacaccgattacttgcgcaaaatggtagaaaccaacccaacggatgtggctgctatcttcctcgagccaatccagggtgaaacgggcgttgttccagcacctgaaggattcctcaaggcagtgcgcgagctgtgcgatgagtacggcatcttgatgatcaccgatgaagtccagactggcgttggccgtaccggcgatttctttgcacatcagcacgatggcgttgttcccgatgtggtgaccatggccaagggacttggcggcggtcttcccatcggtgcttgtttggccactggccgtgcagctgaattgatgaccccaggcaagcacggcaccactttcggtggcaacccagttgcttgtgcagctgccaaggcagtgctgtctgttgtcgatgacgctttctgcgcagaagttgcccgcaagggcgagctgttcaaggaacttcttgccaaggttgacggcgttgtagacgtccgtggcaggggcttgatgttgggcgtggtgctggagcgcgacgtcgcaaagcaagctgttcttgatggttttaagcacggcgttattttgaatgcaccggcggacaacattatccgtttgaccccgccgctggtgatcaccgacgaagaaatcgcagacgcagtcaaggctattgccgagacaatcgcataa

SEQ ID NO: 4 - protein, 391 aa, synthetic construct
MSTLETWPQVIINTYGTPPVELVSGKGATVTDDQGNVYIDLLAGIAVNALGHAHPAIIEAVTNQIGQLGHVSNLFASRPVVEVAEELIKRFSLDDATLAAQTRVFFCNSGAEANEAAFKIARLTGRSRILTAVHGFHGRTMGSLALTGQPDKREAFLPMPSGVEFYPYGDTDYLRKMVETNPTDVAAIFLEPIQGETGVVPAPEGFLKAVRELCDEYGILMITDEVQTGVGRTGDFFAHQHDGVVPDVVTMAKGLGGGLPIGACLATGRAAELMTPGKHGTTFGGNPVACAAAKAVLSVVDDAFCAEVARKGELFKELLAKVDGVVDVRGRGLMLGVVLERDVAKQAVLDGFKHGVILNAPADNIIRLTPPLVITDEEIADAVKAIAETIA

SEQ ID NO: 5 - DNA, 30 bp, synthetic construct
  source 1..30: mol_type = other DNA
tgattacgcccatcgcgcactcggtgttgc

SEQ ID NO: 6 - DNA, 20 bp, synthetic construct
  source 1..20: mol_type = other DNA
catcgcgcactcggtgttgc

SEQ ID NO: 7 - DNA, 20 bp, synthetic construct
  source 1..20: mol_type = other DNA
cgggaacgaccagtcaagcg

SEQ ID NO: 8 - DNA, 20 bp, synthetic construct
  source 1..20: mol_type = other DNA
agtcagaatccgggaacgac

SEQ ID NO: 9 - DNA, 30 bp, synthetic construct
  source 1..30: mol_type = other DNA
gattctgactgcagttcatggtttccacgg

SEQ ID NO: 10 - DNA, 20 bp, synthetic construct
  source 1..20: mol_type = other DNA
gcagttcatggtttccacgg

SEQ ID NO: 11 - DNA, 20 bp, synthetic construct
  source 1..20: mol_type = other DNA
gcgtcatcgacaacagacag

SEQ ID NO: 12 - DNA, 20 bp, synthetic construct
  source 1..20: mol_type = other DNA
tgcgcagaaagcgtcatcga